European Patent Application EP 4 596 686 A1, published August 6, 2025. Title: Method of searching functional molecule causing cellular response. Applicant: KEIO UNIVERSITY. The sequence listing filed with the application follows.

SEQUENCE LISTING (71 sequences)

SEQ ID NO: 1 - DNA, 57 bp, synthetic construct
  source 1..57: mol_type = other DNA
gttaagccagccccgacacaataaaatatctttattttcattacatctgtgtgttgg

SEQ ID NO: 2 - DNA, 40 bp, synthetic construct
  source 1..40: mol_type = other DNA
ctttgtacaagaaagctgggtctaatcgccatcttccagc

SEQ ID NO: 3 - DNA, 40 bp, synthetic construct
  source 1..40: mol_type = other DNA
gctggaagatggcgattagacccagctttcttgtacaaag

SEQ ID NO: 4 - DNA, 42 bp, synthetic construct
  source 1..42: mol_type = other DNA
cactgacgggcaccggagccgcgttaattaataccacatttg

SEQ ID NO: 5 - DNA, 34 bp, synthetic construct
  source 1..34: mol_type = other DNA
gtattaattaacgcggctccggtgcccgtcagtg

SEQ ID NO: 6 - DNA, 45 bp, synthetic construct
  source 1..45: mol_type = other DNA
gaatcatgggaaataggccctctaccacatttgtagaggttttac

SEQ ID NO: 7 - DNA, 45 bp, synthetic construct
  source 1..45: mol_type = other DNA
gtaaaacctctacaaatgtggtagagggcctatttcccatgattc

SEQ ID NO: 8 - DNA, 39 bp, synthetic construct
  source 1..39: mol_type = other DNA
ctatgcggcatcagagcaggatctccataagagaagagg

SEQ ID NO: 9 - DNA, 39 bp, synthetic construct
  source 1..39: mol_type = other DNA
cctcttctcttatggagatcctgctctgatgccgcatag

SEQ ID NO: 10 - DNA, 39 bp, synthetic construct
  source 1..39: mol_type = other DNA
gaaaataaagatattttattgtgtcggggctggcttaac

SEQ ID NO: 11 - DNA, 88 bp, synthetic construct
  source 1..88: mol_type = other DNA
aagttgatgatatcgaattcaaaaagaagctatgttcgccattactcgagtaatggcgaacatagcttcccggtgtttcgtcctttcc

SEQ ID NO: 12 - DNA, 90 bp, synthetic construct
  source 1..90: mol_type = other DNA
aagttgatgatatcgaattcaaaaagccaacgatgtgaagaaattctcgagaatttcttcacatcgttggcccggtgtttcgtcctttcc

SEQ ID NO: 13 - DNA, 88 bp, synthetic construct
  source 1..88: mol_type = other DNA
aagttgatgatatcgaattcaaaaaaagctatgttcgccattaactcgagttaatggcgaacatagcttccggtgtttcgtcctttcc

SEQ ID NO: 14 - DNA, 88 bp, synthetic construct
  source 1..88: mol_type = other DNA
aagttgatgatatcgaattcaaaaagcagtgatgtcctggataactcgagttatccaggacatcactgcccggtgtttcgtcctttcc

SEQ ID NO: 15 - DNA, 32 bp, synthetic construct
  source 1..32: mol_type = other DNA
tttttgaattcgatatcatcaactttgtatag

SEQ ID NO: 16 - DNA, 26 bp, synthetic construct
  source 1..26: mol_type = other DNA
cagttaggccagagaaatgttctggc

SEQ ID NO: 17 - DNA, 20 bp, synthetic construct
  source 1..20: mol_type = other DNA
ggctgtccccagtgcaagtg

SEQ ID NO: 18 - DNA, 22 bp, synthetic construct
  source 1..22: mol_type = other DNA
ggtggctttaccaacagtaccg

SEQ ID NO: 19 - DNA, 19 bp, synthetic construct
  source 1..19: mol_type = other DNA
gctcgacttccagcttggc

SEQ ID NO: 20 - DNA, 27 bp, synthetic construct
  source 1..27: mol_type = other DNA
atttcaggtgtcgtgacaagtttgtac

SEQ ID NO: 21 - DNA, 20 bp, synthetic construct
  source 1..20: mol_type = other DNA
tccctagcaaactggggcac

SEQ ID NO: 22 - DNA, 20 bp, synthetic construct
  source 1..20: mol_type = other DNA
gaagtggtggttgttcacgg

SEQ ID NO: 23 - DNA, 22 bp, synthetic construct
  source 1..22: mol_type = other DNA
tcaggaagcttggatcaaccgg

SEQ ID NO: 24 - DNA, 20 bp, synthetic construct
  source 1..20: mol_type = other DNA
tgatcggtgatcctggaccg

SEQ ID NO: 25 - DNA, 20 bp, synthetic construct
  source 1..20: mol_type = other DNA
ggccagcttggcacttgatg

SEQ ID NO: 26 - DNA, 20 bp, synthetic construct
  source 1..20: mol_type = other DNA
ggacgtgaagaatgtgcgag

SEQ ID NO: 27 - DNA, 20 bp, synthetic construct
  source 1..20: mol_type = other DNA
gagggcgacttaaccttagg

SEQ ID NO: 28 - DNA, 20 bp, synthetic construct
  source 1..20: mol_type = other DNA
aatttcttcacatcgttggc

SEQ ID NO: 29 - DNA, 19 bp, synthetic construct
  source 1..19: mol_type = other DNA
ttatccaggacatcactgc

SEQ ID NO: 30 - DNA, 42 bp, synthetic construct
  source 1..42: mol_type = other DNA
gttaagccagccccgacactgttcacgtagaggaggttatcc

SEQ ID NO: 31 - DNA, 39 bp, synthetic construct
  source 1..39: mol_type = other DNA
ctatgcggcatcagagcaggtaccgttatatgccggcgg

SEQ ID NO: 32 - DNA, 35 bp, synthetic construct
  source 1..35: mol_type = other DNA
cggtgtttcgtcctttccacaagatatataaagcc

SEQ ID NO: 33 - DNA, 32 bp, synthetic construct
  source 1..32: mol_type = other DNA
tagtacagtagtaatagtatatgtgatggatc

SEQ ID NO: 34 - DNA, 126 bp, synthetic construct
  source 1..126: mol_type = other DNA
tcttggctttatatatcttgtggaaaggacgaaacaccggccagctaagtatcaaaggaaactcgagtttcctttgatacttagctggttttttagtacagtagtaatagtatatgtgatggatct

SEQ ID NO: 35 - DNA, 126 bp, synthetic construct
  source 1..126: mol_type = other DNA
tcttggctttatatatcttgtggaaaggacgaaacaccggcctggatttgtggttacgttactcgagtaacgtaaccacaaatccaggttttttagtacagtagtaatagtatatgtgatggatct

SEQ ID NO: 36 - DNA, 126 bp, synthetic construct
  source 1..126: mol_type = other DNA
tcttggctttatatatcttgtggaaaggacgaaacaccgggtgtcctatatccagtgtaaactcgagtttacactggatataggacacttttttagtacagtagtaatagtatatgtgatggatct

SEQ ID NO: 37 - DNA, 126 bp, synthetic construct
  source 1..126: mol_type = other DNA
tcttggctttatatatcttgtggaaaggacgaaacaccggcgtggtgtcaaggtgtactaactcgagttagtacaccttgacaccacgttttttagtacagtagtaatagtatatgtgatggatct

SEQ ID NO: 38 - DNA, 126 bp, synthetic construct
  source 1..126: mol_type = other DNA
tcttggctttatatatcttgtggaaaggacgaaacaccggcgtgtacctttggaggaattactcgagtaattcctccaaaggtacacgttttttagtacagtagtaatagtatatgtgatggatct

SEQ ID NO: 39 - DNA, 126 bp, synthetic construct
  source 1..126: mol_type = other DNA
tcttggctttatatatcttgtggaaaggacgaaacaccggcctaagtatcagaaacttctactcgagtagaagtttctgatacttaggttttttagtacagtagtaatagtatatgtgatggatct

SEQ ID NO: 40 - DNA, 126 bp, synthetic construct
  source 1..126: mol_type = other DNA
tcttggctttatatatcttgtggaaaggacgaaacaccggcctggtagtatgccctacaatctcgagattgtagggcatactaccaggttttttagtacagtagtaatagtatatgtgatggatct

SEQ ID NO: 41 - DNA, 126 bp, synthetic construct
  source 1..126: mol_type = other DNA
tcttggctttatatatcttgtggaaaggacgaaacaccggcctcaaatacaagccactattctcgagaatagtggcttgtatttgaggttttttagtacagtagtaatagtatatgtgatggatct

SEQ ID NO: 42 - DNA, 126 bp, synthetic construct
  source 1..126: mol_type = other DNA
tcttggctttatatatcttgtggaaaggacgaaacaccggcgtgacttcatagaggagtatctcgagatactcctctatgaagtcacgttttttagtacagtagtaatagtatatgtgatggatct

SEQ ID NO: 43 - DNA, 126 bp, synthetic construct
  source 1..126: mol_type = other DNA
tcttggctttatatatcttgtggaaaggacgaaacaccgggctcagatgataacttctgtactcgagtacagaagttatcatctgagcttttttagtacagtagtaatagtatatgtgatggatct

SEQ ID NO: 44 - DNA, 126 bp, synthetic construct
  source 1..126: mol_type = other DNA
tcttggctttatatatcttgtggaaaggacgaaacaccggagttagagacatgggtaatacctcgaggtattacccatgtctctaactttttttagtacagtagtaatagtatatgtgatggatct

SEQ ID NO: 45 - DNA, 23 bp, synthetic construct
  source 1..23: mol_type = other DNA
tgttcacgtagaggaggttatcc

SEQ ID NO: 46 - DNA, 20 bp, synthetic construct
  source 1..20: mol_type = other DNA
gtaccgttatatgccggcgg

SEQ ID NO: 47 - DNA, 24 bp, synthetic construct
  source 1..24: mol_type = other DNA
ccggtgtttcgtcctttccacaag

SEQ ID NO: 48 - DNA, 32 bp, synthetic construct; identical to SEQ ID NO: 33
  source 1..32: mol_type = other DNA

SEQ ID NO: 49 - DNA, 22 bp, synthetic construct
  source 1..22: mol_type = other DNA
gtctcctctgacttcaacagcg

SEQ ID NO: 50 - DNA, 22 bp, synthetic construct
  source 1..22: mol_type = other DNA
accaccctgttgctgtagccaa

SEQ ID NO: 51 - DNA, 20 bp, synthetic construct
  source 1..20: mol_type = other DNA
ctggctttggtgaactgttg

SEQ ID NO: 52 - DNA, 20 bp, synthetic construct
  source 1..20: mol_type = other DNA
agttgctcacagccaagaca

SEQ ID NO: 53 - DNA, 20 bp, synthetic construct
  source 1..20: mol_type = other DNA
gaaacagtgctcgggttttc

SEQ ID NO: 54 - DNA, 20 bp, synthetic construct
  source 1..20: mol_type = other DNA
tagctctgcatggagctgaa

SEQ ID NO: 55 - DNA, 24 bp, synthetic construct
  source 1..24: mol_type = other DNA
tgatcaaccgtggttacaagcagg

SEQ ID NO: 56 - DNA, 23 bp, synthetic construct
  source 1..23: mol_type = other DNA
ctggactgtacctcgttgtacgg

SEQ ID NO: 57 - DNA, 23 bp, synthetic construct
  source 1..23: mol_type = other DNA
ggcctatttcccatgattccttc

SEQ ID NO: 58 - DNA, 28 bp, synthetic construct
  source 1..28: mol_type = other DNA
ccaagaaattattactttctacgtcacg

SEQ ID NO: 59 - DNA, 22 bp, synthetic construct
  source 1..22: mol_type = other DNA
aaagccatacgggaagcaatag

SEQ ID NO: 60 - DNA, 30 bp, synthetic construct
  source 1..30: mol_type = other DNA
aatagggccggtggaaaggacgaaacaccg

SEQ ID NO: 61 - DNA, 31 bp, synthetic construct
  source 1..31: mol_type = other DNA
tgactcgtcgccagttcctacattcgctctc

SEQ ID NO: 62 - DNA, 30 bp, synthetic construct
  source 1..30: mol_type = other DNA
caacggctacgtggaaaggacgaaacaccg

SEQ ID NO: 63 - DNA, 31 bp, synthetic construct
  source 1..31: mol_type = other DNA
ctccatgttgccagttcctacattcgctctc

SEQ ID NO: 64 - DNA, 30 bp, synthetic construct
  source 1..30: mol_type = other DNA
cagcgaatgcgtggaaaggacgaaacaccg

SEQ ID NO: 65 - DNA, 31 bp, synthetic construct
  source 1..31: mol_type = other DNA
ctacaaggatccagttcctacattcgctctc

SEQ ID NO: 66 - DNA, 31 bp, synthetic construct
  source 1..31: mol_type = other DNA
agatccatcacatatactattactactgtac

SEQ ID NO: 67 - DNA, 20 bp, synthetic construct
  source 1..20: mol_type = other DNA
tgcgactgacggttgcaacg

SEQ ID NO: 68 - DNA, 19 bp, synthetic construct
  source 1..19: mol_type = other DNA
agtgtctaagcttggccgc

SEQ ID NO: 69 - DNA, 21 bp, synthetic construct
  source 1..21: mol_type = other DNA
ggatatcaagatctggcctcg

SEQ ID NO: 70 - DNA, 19 bp, synthetic construct
  source 1..19: mol_type = other DNA
gggcccatggtggctttac

SEQ ID NO: 71 - DNA, 21 bp, synthetic construct
  source 1..21: mol_type = other DNA
cttggcaatccggtactgttg